European Patent Application EP 4 714 976 A1, published March 25, 2026. Title: 一种抗FGFR2抗体及其应用. Applicant: 广东东阳光药业股份有限公司. The sequence listing filed with the application follows.

SEQUENCE LISTING (198 sequences)

SEQ ID NO: 1 - protein, 5 aa, synthetic construct
TYNVH

SEQ ID NO: 2 - protein, 5 aa, synthetic construct
NYYIH

SEQ ID NO: 3 - protein, 5 aa, synthetic construct
DYYIH

SEQ ID NO: 4 - protein, 5 aa, synthetic construct
TYNMH

SEQ ID NO: 5 - protein, 5 aa, synthetic construct
SYNLH

SEQ ID NO: 6 - protein, 5 aa, synthetic construct
FYNVH

SEQ ID NO: 7 - protein, 5 aa, synthetic construct
IYNIH

SEQ ID NO: 8 - protein, 5 aa, synthetic construct
FYNIH

SEQ ID NO: 9 - protein, 5 aa, synthetic construct
YYNMH

SEQ ID NO: 10 - protein, 5 aa, synthetic construct
PYNIH

SEQ ID NO: 11 - protein, 5 aa, synthetic construct
TYNIH

SEQ ID NO: 12 - protein, 5 aa, synthetic construct
FYNMH

SEQ ID NO: 13 - protein, 5 aa, synthetic construct
YYNVH

SEQ ID NO: 14 - protein, 17 aa, synthetic construct
SIYPDNGDTSYNQNFKG

SEQ ID NO: 15 - protein, 17 aa, synthetic construct
AIYPDNGDTSYNQRFRV

SEQ ID NO: 16 - protein, 17 aa, synthetic construct
AIYPDNGDTSYNQKFKV

SEQ ID NO: 17 - protein, 17 aa, synthetic construct
AIYPDNGDTFYNRKFKD

SEQ ID NO: 18 - protein, 17 aa, synthetic construct
LIYPENGDTSYNQKFKG

SEQ ID NO: 19 - protein, 17 aa, synthetic construct
LIYPDNGDTSYNQKFKA

SEQ ID NO: 20 - protein, 17 aa, synthetic construct
LIYPDNGDTSYNQKFKG

SEQ ID NO: 21 - protein, 17 aa, synthetic construct
LIYPENGDTSYNQKFKD

SEQ ID NO: 22 - protein, 17 aa, synthetic construct
LIYPDNGDTSYNQKFTG

SEQ ID NO: 23 - protein, 5 aa, synthetic construct
GDFAY

SEQ ID NO: 24 - protein, 5 aa, synthetic construct
GGFDY

SEQ ID NO: 25 - protein, 5 aa, synthetic construct
GGLDY

SEQ ID NO: 26 - protein, 4 aa, synthetic construct
AFTY

SEQ ID NO: 27 - protein, 11 aa, synthetic construct
KASQGVSNDVA

SEQ ID NO: 28 - protein, 11 aa, synthetic construct
GASENIYGALN

SEQ ID NO: 29 - protein, 11 aa, synthetic construct
GASENLYGALN

SEQ ID NO: 30 - protein, 11 aa, synthetic construct
RASENIYSNLA

SEQ ID NO: 31 - protein, 11 aa, synthetic construct
KASQDVSTAVA

SEQ ID NO: 32 - protein, 11 aa, synthetic construct
KASQNVGTNVA

SEQ ID NO: 33 - protein, 11 aa, synthetic construct
RASENIYSYLA

SEQ ID NO: 34 - protein, 11 aa, synthetic construct
KASQDVNTDVS

SEQ ID NO: 35 - protein, 15 aa, synthetic construct
KASQSVDYDGDSYMN

SEQ ID NO: 36 - protein, 11 aa, synthetic construct
KASQDVNTDVA

SEQ ID NO: 37 - protein, 11 aa, synthetic construct
QATQDIVKNLN

SEQ ID NO: 38 - protein, 11 aa, synthetic construct
RASGNIHNYLA

SEQ ID NO: 39 - protein, 7 aa, synthetic construct
SASYRYT

SEQ ID NO: 40 - protein, 7 aa, synthetic construct
GATNLAD

SEQ ID NO: 41 - protein, 7 aa, synthetic construct
NAKTLAD

SEQ ID NO: 42 - protein, 7 aa, synthetic construct
SASYRYS

SEQ ID NO: 43 - protein, 7 aa, synthetic construct
NAKTLAE

SEQ ID NO: 44 - protein, 7 aa, synthetic construct
AATNLAD

SEQ ID NO: 45 - protein, 7 aa, synthetic construct
GISNRFS

SEQ ID NO: 46 - protein, 7 aa, synthetic construct
YATELAE

SEQ ID NO: 47 - protein, 9 aa, synthetic construct
QQHSTTPYT

SEQ ID NO: 48 - protein, 9 aa, synthetic construct
QNVLSTPYT

SEQ ID NO: 49 - protein, 9 aa, synthetic construct
QHFWSTPYT

SEQ ID NO: 50 - protein, 9 aa, synthetic construct
QQHYSTPYT

SEQ ID NO: 51 - protein, 9 aa, synthetic construct
QQHYNTPYT

SEQ ID NO: 52 - protein, 9 aa, synthetic construct
QHHYGTPYT

SEQ ID NO: 53 - protein, 9 aa, synthetic construct
QQHYSTPFT

SEQ ID NO: 54 - protein, 9 aa, synthetic construct
QHFWSTPFT

SEQ ID NO: 55 - protein, 9 aa, synthetic construct
QHFWGTPYT

SEQ ID NO: 56 - protein, 9 aa, synthetic construct
LQGTHQPYT

SEQ ID NO: 57 - protein, 9 aa, synthetic construct
LQFYEFPLT

SEQ ID NO: 58-59 - skipped (2 entries)

SEQ ID NO: 60 - protein, 17 aa, synthetic construct
  PEPTIDE 10: note = The X at position 10 is S or F.
  PEPTIDE 13: note = The X at position 13 is Q or R.
  PEPTIDE 14: note = The X at position 14 is K or R.
  PEPTIDE 16: note = The X at position 16 is K, R or T.
  PEPTIDE 17: note = The X at position 17 is V, D, G or A.
AIYPDNGDTXYNXXFXX

SEQ ID NO: 61 - protein, 17 aa, synthetic construct
  PEPTIDE 5: note = The X at position 5 is D or E.
  PEPTIDE 16: note = The X at position 16 is K, R or T.
  PEPTIDE 17: note = The X at position 17 is V, D, G or A.
LIYPXNGDTSYNQKFXX

SEQ ID NO: 62 - skipped

SEQ ID NO: 63 - protein, 114 aa, synthetic construct [sequence omitted]

SEQ ID NO: 64 - protein, 113 aa, synthetic construct
EIQLQQSGAELVKPGASVKMSCKASGYIFRNYYIHWVKRTPGQGLEWIGAIYPDNGDTSYNQRFKVKATLTADTSSSTAYMQLSSLTSEDSAVYYCARAFTYWGQGTTLTVSS

SEQ ID NO: 65 - protein, 113 aa, synthetic construct
QVQLQQPGAEVVKPGASVKMSCKASGYTFTDYYIHWVKQTPGQGLEWIGAIYPDNGDTSYNQKFKVKATLTADKSSSTAYMQLSSLTSEDSAVYYCARAFTYWGQGTLVTVSA

SEQ ID NO: 66 - protein, 114 aa, synthetic construct
QVQLQQSGAELVKPGASVKMSCKASGYTFTIYNIHWVRQTPGQGLEWIGLIYPDNGDTSYNQKFKAKATLTADKSSSTAYMQLSSLTSEDSAVYYCARGGFDYWGQGTSLTVSS

SEQ ID NO: 67 - protein, 114 aa, synthetic construct
EVQLQQSGPELVKPGASVKMSCKASGYTFATYNMHWVKQTTGQGLEWIGAIYPDNGDTFYNRKFKDKATLTADKSSTTAYMQLSSLTSEDSAVYYCARGDFAYWGQGTLVTVSA

SEQ ID NO: 68 - protein, 114 aa, synthetic construct
EVQLQQSGAELVKPGASVKMSCKASGYTFASYNLHWVKQTPGQGLEWIGLIYPENGDTSYNQKFKGKATLTADKSSSTAYIQLSSLTSEDSAVYFCARGGFDYWGQGTSLTVSS

SEQ ID NO: 69 - protein, 114 aa, synthetic construct
EVQLQQSGAELVKPGASVKMSCKASGYTFSFYNVHWVRQTPGQGLEWIGLIYPDNGDTSYNQKFKAKATLTADKSSSAAYMQLSSLTSEDSAVYYCARGGFDYWGQGTSLTVSS

SEQ ID NO: 70 - protein, 114 aa, synthetic construct
QVQLQQSGAELVKPGASVKMSCKASGYTFTIYNIHWVRQTPGQGLEWIGLIYPDNGDTSYNQKFKAKATLTADKSSSTAYMQLSSLTSEDSAVYYCARGGFDYWGQGTTLTVSS

SEQ ID NO: 71 - protein, 114 aa, synthetic construct
EVQLQQSGAELVKPGASVKMSCKASGYTFSFYNIHWVRQTPGQGLEWIGLIYPDNGDTSYNQKFKAKATLTADKSSSTAYMQLSSLTSEDSAVYYCARGGFDYWGQGTTLTVSS

SEQ ID NO: 72 - protein, 114 aa, synthetic construct
QVQLQQSGAELVKPGASVKMSCKASGYTFSFYNIHWVRQTPGQGLEWIGLIYPDNGDTSYNQKFKAKATLTADKSSSTAYMQLSSLTSEDSAVYYCARGGFDYWGQGTTLTVSS

SEQ ID NO: 73 - protein, 114 aa, synthetic construct
EVQLQQSGAELVKPGASVKMSCKASGYTFRYYNMHWVKRTPGQGLEWIGLIYPDNGDTSYNQKFKGKATLTADTSSSTAYMQLSSLTSEDSAVYYCARGGFDYWGQGTTLTVSS

SEQ ID NO: 74 - protein, 114 aa, synthetic construct
QVQLQQSGAELVKPGASVKMSCKASGYTFAPYNIHWVRQTPGQGLEWIGLIYPDNGDTSYNQKFKAKATLTADKSSSTAYMQLSSLTSEDSAVYYCARGGFDYWGQGTSLTVSS

SEQ ID NO: 75 - protein, 114 aa, synthetic construct
QIQLQQSGAELVKPGASVKMSCKASGYTFASYNLHWVKQTPGQGLEWIGLIYPENGDTSYNQKFKGKATLTADTSSTTAYIQLSSLTSEDSAVYFCARGGFDYWGQGTSLTVSS

SEQ ID NO: 76 - protein, 114 aa, synthetic construct
QVQLQQPGAELVKPGASVKMSCKASGYTFASYNLHWVKQTPGQGLEWIGLIYPENGDTSYNQKFKGKATLTADKSSSTAYIQLSSLTSEDSAVYFCARGGFDYWGQGTTLTVSQ

SEQ ID NO: 77 - protein, 114 aa, synthetic construct
QLQLQQSGAELVKPGASVKMSCKASGYTFASYNLHWVKQTPGQGLEWIGLIYPENGDTSYNQKFKDKATLTADKSSTTAYIQLSSLASEDSAVYFCARGGFDYWGQGTTLTVSS

SEQ ID NO: 78 - protein, 114 aa, synthetic construct
QVQLQQSGAELVKPGASVKMSCKASGYTFTTYNIHWVRQTPGQGLEWIGLIYPDNGDTSYNQKFKAKATLTADKSSSTAYMHLSSLTSEDSAVYYCARGGFDYWGQGTTLTVSS

SEQ ID NO: 79 - protein, 114 aa, synthetic construct
EIQLQQSGAELVKPGASVKMSCKASGYIFRYYNMHWVKRTPGQGLEWIGLIYPDNGDTSYNQKFKGKATLTADTSSSTAYMQLSSLTSEDSAVYYCARGGLDYWGQGTTLTVSS

SEQ ID NO: 80 - protein, 114 aa, synthetic construct
QVQLQQSGAELVKPGASVKMSCKASGYTFRYYNMHWVKRTPGQGLEWIGLIYPDNGDTSYNQKFKGKATLTADTSSSTAYMQLSSLTSEDSAVYYCARGGLDYWGQGTSLTVSS

SEQ ID NO: 81 - protein, 114 aa, synthetic construct
EIQLQQSGAELVKPGASVKMSCKASGYTFSFYNMHWVKRTPGQGLEWIGLIYPDNGDTSYNQKFKGKATLTADTSSSTAYMQLSSLTSEDSAVYYCARGGLDYWGQGTSLTVSS

SEQ ID NO: 82 - protein, 114 aa, synthetic construct
QVQLQQPGAVLVKPGASVRMSCKASGYTFPYYNVHWVKRTPGQGLEWIGLIYPDNGDTSYNQKFTGKATLTADTSSSTAYMQLSSLTSEDSAVYYCARGGLDYWGQGTTLTVSA

SEQ ID NO: 83 - protein, 114 aa, synthetic construct
EIQLQQSGAELVKPGASVKMSCKASGYTFRYYNMHWVKRTPGQGLEWIGLIYPDNGDTSYNQKFKGKATLTADTSSSTAYMQLSSLTSEDSAVYYCARGGLDYWGQGTTLTVSS

SEQ ID NO: 84 - protein, 114 aa, synthetic construct
EIQLQQSGAELVKPGASVKMSCKASGYTFSFYNMHWVKRTPGQGLEWIGLIYPDNGDTSYNQKFKGKATLTADTSSSTAYMQLSSLTSEDSAVYYCARGGLDYWGQGTTLTVSS

SEQ ID NO: 85 - protein, 114 aa, synthetic construct
EVQLQQSGADLVKPGASVKMSCKASGYTFSYYNMHWVRRTPGQGLEWIGLIYPDNGDTSYNQKFKGKATLTADTSSSTAYMQLSSLTSEDSAVYYCARGGLDYWGQGTTLTVSS

SEQ ID NO: 86 - protein, 114 aa, synthetic construct
QVQLQQSGAELVKPGASVKMSCKASGYTFSFYNMHWVKRTPGRGLEWIGLIYPDNGDTSYNQKFKGKATLTADTSSSTAYMQLSSLTSEDSAVYYCARGGLDYWGQGTSLTVSS

SEQ ID NO: 87 - protein, 114 aa, synthetic construct
EIQLQQSGAELVKPGASVKMSCKASGYTFRYYNMHWVKRTPGQGLEWIGLIYPDNGDTSYNQKFKGKATLTADTSSSTAYMQLSSLTSEDSAVYYCARGGLDYWGQGTSLTVSS

SEQ ID NO: 88 - protein, 114 aa, synthetic construct
QIQLQQSGAELVKPGASVKMSCKASGYTFRYYNMHWVKRTPGQGLEWIGLIYPDNGDTSYNQKFKGKATLTADTSSSTAYMQLSSLTSEDSAVYYCARGGLDYWGQGTSLTVSS

SEQ ID NO: 89 - protein, 114 aa, synthetic construct; identical to SEQ ID NO: 80

SEQ ID NO: 90 - protein, 107 aa, synthetic construct [sequence omitted]

SEQ ID NO: 91 - protein, 107 aa, synthetic construct
DILMTQSPASLSASVGETVTIKCGASENIYGALNWYQRKQGKSPQLLIYGATNLADGMSSRFSGSGSGRQYSLKISSLHPDDVATYYCQNVLSTPYTFGGGTKLEIK

SEQ ID NO: 92 - protein, 107 aa, synthetic construct
DILITQSPASLSASVGETVTITCGASENIYGALNWYQRKQGKSPQLLIYGATNLADGMSSRFSGSGSGRQYSLKISSLHPDDVATYYCQNVLSTPYTFGGGTKLEIK

SEQ ID NO: 93 - protein, 107 aa, synthetic construct
DIVMTQSQKFMSTSVGDRVSVTCKASQNVGTNVAWYQQKPGQSPKALIYSASYRYSGVPDRFTGSGSGTDFTLTISNVQAEDLADYFCQQHYSTPYTFGGGTKLEMK

SEQ ID NO: 94 - protein, 107 aa, synthetic construct
DVLMTQSPASLSASVGETVTITCGASENIYGALNWYQRKQGKSPQLLIYGATNLADGMSSRFSGSGSGRQYSLKISSLHPDDVATYYCQNVLSTPYTFGGGTKLEMK

SEQ ID NO: 95 - protein, 107 aa, synthetic construct
DIQMIQSPASLSVSVGETVTITCRASENIYSNLAWYQQKQGKSPQLLVYNAKTLADGVPSRFSGSGSGTQYSLKINSLQPEDFGSYYCQHFWSTPYTFGGGTKLEIK

SEQ ID NO: 96 - protein, 107 aa, synthetic construct
DIVMTQSHKFMSTSVGDRVNITCKASQDVSTAVAWYQQKPGQSPKLLIYSASYRYSGVPDRFTGSGSGTDFTFTISSVQAEDLAVYYCQQHYSTPYTFGGGTKLEMK

SEQ ID NO: 97 - protein, 107 aa, synthetic construct
NIVMTQSQKFMSTSVGDRVSVTCKASQNVGTNVAWYQQKPGQSPKALIYSASYRYSGVPDRFTGSGSGTDFTLTISGVQAEDLADYYCQQHYNTPYTFGGGTKLEIK

SEQ ID NO: 98 - protein, 107 aa, synthetic construct
DVLMTQSPASLSASVGETVTITCGASENIYGALNWYQRKQGKSPQLLIYGATNLADGMSSRFSGSGSGRQYSLKISSLHPDDVATYYCQNVLSTPYTFGGGTKLEIK

SEQ ID NO: 99 - protein, 107 aa, synthetic construct
DIQMTQSPASLSASVGETVTITCRASENIYSYLAWYQQKQGKSPQLLVYNAKTLAEGVPSRFSGSGSGTQFSLKINSLQPEDFGSYYCQHHYGTPYTFGGGTKLEMK

SEQ ID NO: 100 - protein, 107 aa, synthetic construct
DIQMTQSPASLSASVGETVTITCGASENIYGALNWYQRKQGKSPQLLIYGATNLADGMSSRFSGSGSGRQYSLKISSLHPDDVATYYCQNVLSTPYTFGGGTKLELK

SEQ ID NO: 101 - protein, 107 aa, synthetic construct
DIVMTQSQKFMSTSVGDRVSVTCKASQNVGTNVAWYQQKPGQSPKALIYSASYRYSGVPDRFTGSGSGTDFTLTISNVQSEDLAEYFCQQHYSTPFTFGSGTKLEIK

SEQ ID NO: 102 - protein, 107 aa, synthetic construct
DIKMTQSPASLSASVGETVTITCGASENIYGALNWYQRKQGKSPQLLIYGATNLADGMSSRFSGSGSGRQYSLKISSLHPDDVATYYCQNVLSTPYTFGGGTKLEIK

SEQ ID NO: 103 - protein, 107 aa, synthetic construct
DIQMTQSPASLSASVGETVTITCGASENIYGALNWYQRKQGKSPQLLIYGATNLADGMSSRFSGSGSGRQYSLKISSLHPDDVATYYCQNVLSTPYTFGGGTKLEIK

SEQ ID NO: 104 - protein, 107 aa, synthetic construct
DIVMTQSQKFMSTSVGDRVSVTCKASQNVGTNVAWYQQKPGQSPKALIYSASYRYSGVPDRFTGSGSGTDYTLTISSVQAEDLALYYCQQHYSTPYTFGGGTKLELK

SEQ ID NO: 105 - protein, 107 aa, synthetic construct
DIVMTQSHKFMSTSVGDRVSITCKASQDVNTDVSWYQQKPGQSPKLLIYSASYRYTGVPTRFTGSGSGTDFTFTISGVQAEDLADYYCQQHYNTPYTFGGGTRLEIK

SEQ ID NO: 106 - protein, 107 aa, synthetic construct
DIQMIQSPASLSASVGETVTITCGASENIYGALNWYQRKQGKSPQLLIYGATNLADGMSSRFSGSGSGRQYSLKISSLHPDDVATYYCQNVLSTPYTFGGGTKLEIK

SEQ ID NO: 107 - protein, 107 aa, synthetic construct
DIQMTQSPASLSVSVGETVTITCRASENIYSNLAWYQQKQGKSPQLLVYNAKTLADGVPSRFSGSGSGTQYSLKINSLQPEDFGSYYCQHFWSTPFTFGSGTKLELK

SEQ ID NO: 108 - protein, 107 aa, synthetic construct
NIVMTQSQKFMSTSVGDRVSVTCKASQNVGTNVAWYQQKPGQSPKALIYSASYRYTGVPDRFTGSGSGTDFTFTISSVQAEDLAVYYCQQHYSTPYTFGGGTKLEIK

SEQ ID NO: 109 - protein, 107 aa, synthetic construct
DVQITQSPASLSASVGETVTITCGASENIYGALNWYQRKQGKSPQLLIYGATNLADGMSSRFSGSGSGRQYSLKISSLHPDDVATYYCQNVLSTPYTFGGGTKLEIK

SEQ ID NO: 110 - protein, 107 aa, synthetic construct
DIVLTQSPASLSASVGETVTITCGASENIYGALNWYQRKQGKSPQLLIYGATNLADGMSSRFSGSGSGRQYSLKISSLHPDDVATYYCQNVLSTPYTFGGGTKLEIK

SEQ ID NO: 111 - protein, 107 aa, synthetic construct
DIVLTQSPASLSVSVGETVTITCRASENIYSNLAWYQQKQGKSPQLLVYAATNLADGVPSRFSGSGSGTQYSLKINSLQSEDFGSYYCQHFWGTPYTFGGGTKLELK

SEQ ID NO: 112 - protein, 107 aa, synthetic construct
DIQMIQSPASMSASVGETVTITCGASENIYGALNWYQRKQGKSPQLLIYGATNLADGMSSRFSGSGSGRQYSLKISSLHPDDVATYYCQNVLSTPYTFGGGTKLEMK

SEQ ID NO: 113 - protein, 111 aa, synthetic construct
EIVLTQSPASLAVSLGQRATISCKASQSVDYDGDSYMNWYQQKPGQPPKLLIYGISNRFSGVPDRFSGSGSGTDFTLKISTIKPEDLGMYYCLQGTHQPYTFGGGTKLEIK

SEQ ID NO: 114 - protein, 107 aa, synthetic construct
NIVMTQSHKFMSTSVGDRVSITCKASQDVNTDVAWYQQKPGQSPKLLIYSASYRYTGVPTRFTGSGSGTDFTFTISGVQAEDLADYYCQQHYNTPYTFGGGTKLELK

SEQ ID NO: 115 - protein, 107 aa, synthetic construct
DIQMTQSPSSMSASLGDRITITCQATQDIVKNLNWYQQKPGKPPSFLIYYATELAEGVPSRFSGSGSGSDYSLTISNLESEDFADYYCLQFYEFPLTFGAGTKLELK

SEQ ID NO: 116 - protein, 107 aa, synthetic construct
DIVMTQSPASLSASVGETVTITCRASGNIHNYLAWYQQKQGKSPQLLVYNAKTLADGVPSRFSGSGSGTQYSLKINSLQPEDFGSYYCQHFWSTPYTFGGGTKLEMK

SEQ ID NO: 117 - protein, 330 aa, synthetic construct
ASTKGPSVFPLAPSSKSTSGGTAALGCLVKDYFPEPVTVSWNSGALTSGVHTFPAVLQSSGLYSLSSVVTVPSSSLGTQTYICNVNHKPSNTKVDKKVEPKSCDKTHTCPPCPAPELLGGPSVFLFPPKPKDTLMISRTPEVTCVVVDVSHEDPEVKFNWYVDGVEVHNAKTKPREEQYNSTYRVVSVLTVLHQDWLNGKEYKCKVSNKALPAPIEKTISKAKGQPREPQVYTLPPSREEMTKNQVSLTCLVKGFYPSDIAVEWESNGQPENNYKTTPPVLDSDGSFFLYSKLTVDKSRWQQGNVFSCSVMHEALHNHYTQKSLSLSPGK

SEQ ID NO: 118 - protein, 107 aa, synthetic construct [sequence omitted]

SEQ ID NO: 119 - protein, 4 aa, synthetic construct
GGGS

SEQ ID NO: 120 - protein, 5 aa, synthetic construct
GGGGS

SEQ ID NO: 121 - protein, 10 aa, synthetic construct
GGGGSGGGGS

SEQ ID NO: 122 - protein, 15 aa, synthetic construct
GGGGSGGGGSGGGGS

SEQ ID NO: 123 - protein, 15 aa, synthetic construct
GGGGSGGGGSGDGGS

SEQ ID NO: 124 - protein, 229 aa, synthetic construct
ESKYGPPCPSCPAPEFLGGPSVFLFPPKPKDTLMISRTPEVTCVVVDVSQEDPEVQFNWYVDGVEVHNAKTKPREEQFNSTYRVVSVLTVLHQDWLNGKEYKCKVSNKGLPSSIEKTISKAKGQPREPQVYTLPPSQEEMTKNQVSLTCLVKGFYPSDIAVEWESNGQPENNYKTTPPVLDSDGSFFLYSRLTVDKSRWQEGNVFSCSVMHEALHNHYTQKSLSLSLGK

SEQ ID NO: 125 - protein, 228 aa, synthetic construct
ESKYGPPCPPCPAPEAAGGPSVFLFPPKPKDTLMISRTPEVTCVVVDVSQEDPEVQFNWYVDGVEVHNAKTKPREEQFNSTYRVVSVLTVLHQDWLNGKEYKCKVSNKGLPSSIEKTISKAKGQPREPQVYTLPPSQEEMTKNQVSLTCLVKGFYPSDIAVEWESNGQPENNYKTTPPVLDSDGSFFLYSKLTVDKSRWQEGNVFSCSVMHEALHNHYTQKSLSLSLG

SEQ ID NO: 126 - skipped

SEQ ID NO: 127 - protein, 6 aa, synthetic construct
  PEPTIDE 6: note = The X at position 6 is S or T.
SASYRX

SEQ ID NO: 128 - skipped

SEQ ID NO: 129 - protein, 9 aa, synthetic construct
  PEPTIDE 2: note = The X at position 2 is N, H or Q.
  PEPTIDE 3: note = The X at position 3 is V, F or H.
  PEPTIDE 4: note = The X at position 4 is L, W or Y.
  PEPTIDE 5: note = The X at position 5 is S, N or G.
  PEPTIDE 8: note = The X at position 8 is Y or F.
QXXXXTPXT

SEQ ID NO: 130 - protein, 9 aa, synthetic construct
  PEPTIDE 3: note = The X at position 3 is G or F.
  PEPTIDE 4: note = The X at position 4 is T or Y.
  PEPTIDE 5: note = The X at position 5 is H or E.
  PEPTIDE 6: note = The X at position 6 is Q or F.
  PEPTIDE 8: note = The X at position 8 is Y or L.
LQXXXXPXT

SEQ ID NO: 131 - protein, 444 aa, synthetic construct
QVQLVQSGAEVKKPGSSVKVSCKASGYIFTTYNVHWVRQAPGQGLEWIGSIYPDNGDTSYNQNFKGRATITADKSTSTAYMELSSLRSEDTAVYYCARGDFAYWGQGTLVTVSSASTKGPSVFPLAPSSKSTSGGTAALGCLVKDYFPEPVTVSWNSGALTSGVHTFPAVLQSSGLYSLSSVVTVPSSSLGTQTYICNVNHKPSNTKVDKKVEPKSCDKTHTCPPCPAPELLGGPSVFLFPPKPKDTLMISRTPEVTCVVVDVSHEDPEVKFNWYVDGVEVHNAKTKPREEQYNSTYRVVSVLTVLHQDWLNGKEYKCKVSNKALPAPIEKTISKAKGQPREPQVYTLPPSREEMTKNQVSLTCLVKGFYPSDIAVEWESNGQPENNYKTTPPVLDSDGSFFLYSKLTVDKSRWQQGNVFSCSVMHEALHNHYTQKSLSLSPGK

SEQ ID NO: 132 - protein, 214 aa, synthetic construct
DIQMTQSPSSLSASVGDRVTITCKASQGVSNDVAWYQQKPGKAPKLLIYSASYRYTGVPSRFSGSGSGTDFTFTISSLQPEDIATYYCQQHSTTPYTFGQGTKLEIKRTVAAPSVFIFPPSDEQLKSGTASVVCLLNNFYPREAKVQWKVDNALQSGNSQESVTEQDSKDSTYSLSSTLTLSKADYEKHKVYACEVTHQGLSSPVTKSFNRGEC

SEQ ID NO: 133 - protein, 444 aa, synthetic construct
EVQLQQSGAELVKPGASVKMSCKASGYTFSFYNVHWVRQTPGQGLEWIGLIYPDNGDTSYNQKFKAKATLTADKSSSAAYMQLSSLTSEDSAVYYCARGGFDYWGQGTSLTVSSASTKGPSVFPLAPSSKSTSGGTAALGCLVKDYFPEPVTVSWNSGALTSGVHTFPAVLQSSGLYSLSSVVTVPSSSLGTQTYICNVNHKPSNTKVDKKVEPKSCDKTHTCPPCPAPELLGGPSVFLFPPKPKDTLMISRTPEVTCVVVDVSHEDPEVKFNWYVDGVEVHNAKTKPREEQYNSTYRVVSVLTVLHQDWLNGKEYKCKVSNKALPAPIEKTISKAKGQPREPQVYTLPPSREEMTKNQVSLTCLVKGFYPSDIAVEWESNGQPENNYKTTPPVLDSDGSFFLYSKLTVDKSRWQQGNVFSCSVMHEALHNHYTQKSLSLSPGK

SEQ ID NO: 134 - protein, 214 aa, synthetic construct
DIVMTQSHKFMSTSVGDRVNITCKASQDVSTAVAWYQQKPGQSPKLLIYSASYRYSGVPDRFTGSGSGTDFTFTISSVQAEDLAVYYCQQHYSTPYTFGGGTKLEMKRTVAAPSVFIFPPSDEQLKSGTASVVCLLNNFYPREAKVQWKVDNALQSGNSQESVTEQDSKDSTYSLSSTLTLSKADYEKHKVYACEVTHQGLSSPVTKSFNRGEC

SEQ ID NO: 135 - protein, 444 aa, synthetic construct
QVQLQQSGAELVKPGASVKMSCKASGYTFAPYNIHWVRQTPGQGLEWIGLIYPDNGDTSYNQKFKAKATLTADKSSSTAYMQLSSLTSEDSAVYYCARGGFDYWGQGTSLTVSSASTKGPSVFPLAPSSKSTSGGTAALGCLVKDYFPEPVTVSWNSGALTSGVHTFPAVLQSSGLYSLSSVVTVPSSSLGTQTYICNVNHKPSNTKVDKKVEPKSCDKTHTCPPCPAPELLGGPSVFLFPPKPKDTLMISRTPEVTCVVVDVSHEDPEVKFNWYVDGVEVHNAKTKPREEQYNSTYRVVSVLTVLHQDWLNGKEYKCKVSNKALPAPIEKTISKAKGQPREPQVYTLPPSREEMTKNQVSLTCLVKGFYPSDIAVEWESNGQPENNYKTTPPVLDSDGSFFLYSKLTVDKSRWQQGNVFSCSVMHEALHNHYTQKSLSLSPGK

SEQ ID NO: 136 - protein, 214 aa, synthetic construct
DIVMTQSQKFMSTSVGDRVSVTCKASQNVGTNVAWYQQKPGQSPKALIYSASYRYSGVPDRFTGSGSGTDFTLTISNVQSEDLAEYFCQQHYSTPFTFGSGTKLEIKRTVAAPSVFIFPPSDEQLKSGTASVVCLLNNFYPREAKVQWKVDNALQSGNSQESVTEQDSKDSTYSLSSTLTLSKADYEKHKVYACEVTHQGLSSPVTKSFNRGEC

SEQ ID NO: 137 - protein, 444 aa, synthetic construct
EIQLQQSGAELVKPGASVKMSCKASGYIFRYYNMHWVKRTPGQGLEWIGLIYPDNGDTSYNQKFKGKATLTADTSSSTAYMQLSSLTSEDSAVYYCARGGLDYWGQGTTLTVSSASTKGPSVFPLAPSSKSTSGGTAALGCLVKDYFPEPVTVSWNSGALTSGVHTFPAVLQSSGLYSLSSVVTVPSSSLGTQTYICNVNHKPSNTKVDKKVEPKSCDKTHTCPPCPAPELLGGPSVFLFPPKPKDTLMISRTPEVTCVVVDVSHEDPEVKFNWYVDGVEVHNAKTKPREEQYNSTYRVVSVLTVLHQDWLNGKEYKCKVSNKALPAPIEKTISKAKGQPREPQVYTLPPSREEMTKNQVSLTCLVKGFYPSDIAVEWESNGQPENNYKTTPPVLDSDGSFFLYSKLTVDKSRWQQGNVFSCSVMHEALHNHYTQKSLSLSPGK

SEQ ID NO: 138 - protein, 214 aa, synthetic construct
DIQMIQSPASLSASVGETVTITCGASENIYGALNWYQRKQGKSPQLLIYGATNLADGMSSRFSGSGSGRQYSLKISSLHPDDVATYYCQNVLSTPYTFGGGTKLEIKRTVAAPSVFIFPPSDEQLKSGTASVVCLLNNFYPREAKVQWKVDNALQSGNSQESVTEQDSKDSTYSLSSTLTLSKADYEKHKVYACEVTHQGLSSPVTKSFNRGEC

SEQ ID NO: 139 - protein, 444 aa, synthetic construct
QVQLQQSGAELVKPGASVKMSCKASGYTFRYYNMHWVKRTPGQGLEWIGLIYPDNGDTSYNQKFKGKATLTADTSSSTAYMQLSSLTSEDSAVYYCARGGLDYWGQGTSLTVSSASTKGPSVFPLAPSSKSTSGGTAALGCLVKDYFPEPVTVSWNSGALTSGVHTFPAVLQSSGLYSLSSVVTVPSSSLGTQTYICNVNHKPSNTKVDKKVEPKSCDKTHTCPPCPAPELLGGPSVFLFPPKPKDTLMISRTPEVTCVVVDVSHEDPEVKFNWYVDGVEVHNAKTKPREEQYNSTYRVVSVLTVLHQDWLNGKEYKCKVSNKALPAPIEKTISKAKGQPREPQVYTLPPSREEMTKNQVSLTCLVKGFYPSDIAVEWESNGQPENNYKTTPPVLDSDGSFFLYSKLTVDKSRWQQGNVFSCSVMHEALHNHYTQKSLSLSPGK

SEQ ID NO: 140 - protein, 214 aa, synthetic construct
DIQMTQSPASLSVSVGETVTITCRASENIYSNLAWYQQKQGKSPQLLVYNAKTLADGVPSRFSGSGSGTQYSLKINSLQPEDFGSYYCQHFWSTPFTFGSGTKLELKRTVAAPSVFIFPPSDEQLKSGTASVVCLLNNFYPREAKVQWKVDNALQSGNSQESVTEQDSKDSTYSLSSTLTLSKADYEKHKVYACEVTHQGLSSPVTKSFNRGEC

SEQ ID NO: 141 - protein, 444 aa, synthetic construct
EIQLQQSGAELVKPGASVKMSCKASGYTFSFYNMHWVKRTPGQGLEWIGLIYPDNGDTSYNQKFKGKATLTADTSSSTAYMQLSSLTSEDSAVYYCARGGLDYWGQGTSLTVSSASTKGPSVFPLAPSSKSTSGGTAALGCLVKDYFPEPVTVSWNSGALTSGVHTFPAVLQSSGLYSLSSVVTVPSSSLGTQTYICNVNHKPSNTKVDKKVEPKSCDKTHTCPPCPAPELLGGPSVFLFPPKPKDTLMISRTPEVTCVVVDVSHEDPEVKFNWYVDGVEVHNAKTKPREEQYNSTYRVVSVLTVLHQDWLNGKEYKCKVSNKALPAPIEKTISKAKGQPREPQVYTLPPSREEMTKNQVSLTCLVKGFYPSDIAVEWESNGQPENNYKTTPPVLDSDGSFFLYSKLTVDKSRWQQGNVFSCSVMHEALHNHYTQKSLSLSPGK

SEQ ID NO: 142 - protein, 214 aa, synthetic construct
NIVMTQSQKFMSTSVGDRVSVTCKASQNVGTNVAWYQQKPGQSPKALIYSASYRYTGVPDRFTGSGSGTDFTFTISSVQAEDLAVYYCQQHYSTPYTFGGGTKLEIKRTVAAPSVFIFPPSDEQLKSGTASVVCLLNNFYPREAKVQWKVDNALQSGNSQESVTEQDSKDSTYSLSSTLTLSKADYEKHKVYACEVTHQGLSSPVTKSFNRGEC

SEQ ID NO: 143 - protein, 444 aa, synthetic construct
EIQLQQSGAELVKPGASVKMSCKASGYTFSFYNMHWVKRTPGQGLEWIGLIYPDNGDTSYNQKFKGKATLTADTSSSTAYMQLSSLTSEDSAVYYCARGGLDYWGQGTTLTVSSASTKGPSVFPLAPSSKSTSGGTAALGCLVKDYFPEPVTVSWNSGALTSGVHTFPAVLQSSGLYSLSSVVTVPSSSLGTQTYICNVNHKPSNTKVDKKVEPKSCDKTHTCPPCPAPELLGGPSVFLFPPKPKDTLMISRTPEVTCVVVDVSHEDPEVKFNWYVDGVEVHNAKTKPREEQYNSTYRVVSVLTVLHQDWLNGKEYKCKVSNKALPAPIEKTISKAKGQPREPQVYTLPPSREEMTKNQVSLTCLVKGFYPSDIAVEWESNGQPENNYKTTPPVLDSDGSFFLYSKLTVDKSRWQQGNVFSCSVMHEALHNHYTQKSLSLSPGK

SEQ ID NO: 144 - protein, 214 aa, synthetic construct
DIVLTQSPASLSVSVGETVTITCRASENIYSNLAWYQQKQGKSPQLLVYAATNLADGVPSRFSGSGSGTQYSLKINSLQSEDFGSYYCQHFWGTPYTFGGGTKLELKRTVAAPSVFIFPPSDEQLKSGTASVVCLLNNFYPREAKVQWKVDNALQSGNSQESVTEQDSKDSTYSLSSTLTLSKADYEKHKVYACEVTHQGLSSPVTKSFNRGEC

SEQ ID NO: 145 - protein, 444 aa, synthetic construct
EIQLQQSGAELVKPGASVKMSCKASGYTFRYYNMHWVKRTPGQGLEWIGLIYPDNGDTSYNQKFKGKATLTADTSSSTAYMQLSSLTSEDSAVYYCARGGLDYWGQGTSLTVSSASTKGPSVFPLAPSSKSTSGGTAALGCLVKDYFPEPVTVSWNSGALTSGVHTFPAVLQSSGLYSLSSVVTVPSSSLGTQTYICNVNHKPSNTKVDKKVEPKSCDKTHTCPPCPAPELLGGPSVFLFPPKPKDTLMISRTPEVTCVVVDVSHEDPEVKFNWYVDGVEVHNAKTKPREEQYNSTYRVVSVLTVLHQDWLNGKEYKCKVSNKALPAPIEKTISKAKGQPREPQVYTLPPSREEMTKNQVSLTCLVKGFYPSDIAVEWESNGQPENNYKTTPPVLDSDGSFFLYSKLTVDKSRWQQGNVFSCSVMHEALHNHYTQKSLSLSPGK

SEQ ID NO: 146 - protein, 214 aa, synthetic construct
NIVMTQSHKFMSTSVGDRVSITCKASQDVNTDVAWYQQKPGQSPKLLIYSASYRYTGVPTRFTGSGSGTDFTFTISGVQAEDLADYYCQQHYNTPYTFGGGTKLELKRTVAAPSVFIFPPSDEQLKSGTASVVCLLNNFYPREAKVQWKVDNALQSGNSQESVTEQDSKDSTYSLSSTLTLSKADYEKHKVYACEVTHQGLSSPVTKSFNRGEC

SEQ ID NO: 147 - protein, 444 aa, synthetic construct
QIQLQQSGAELVKPGASVKMSCKASGYTFRYYNMHWVKRTPGQGLEWIGLIYPDNGDTSYNQKFKGKATLTADTSSSTAYMQLSSLTSEDSAVYYCARGGLDYWGQGTSLTVSSASTKGPSVFPLAPSSKSTSGGTAALGCLVKDYFPEPVTVSWNSGALTSGVHTFPAVLQSSGLYSLSSVVTVPSSSLGTQTYICNVNHKPSNTKVDKKVEPKSCDKTHTCPPCPAPELLGGPSVFLFPPKPKDTLMISRTPEVTCVVVDVSHEDPEVKFNWYVDGVEVHNAKTKPREEQYNSTYRVVSVLTVLHQDWLNGKEYKCKVSNKALPAPIEKTISKAKGQPREPQVYTLPPSREEMTKNQVSLTCLVKGFYPSDIAVEWESNGQPENNYKTTPPVLDSDGSFFLYSKLTVDKSRWQQGNVFSCSVMHEALHNHYTQKSLSLSPGK

SEQ ID NO: 148 - protein, 214 aa, synthetic construct
DIQMTQSPSSMSASLGDRITITCQATQDIVKNLNWYQQKPGKPPSFLIYYATELAEGVPSRFSGSGSGSDYSLTISNLESEDFADYYCLQFYEFPLTFGAGTKLELKRTVAAPSVFIFPPSDEQLKSGTASVVCLLNNFYPREAKVQWKVDNALQSGNSQESVTEQDSKDSTYSLSSTLTLSKADYEKHKVYACEVTHQGLSSPVTKSFNRGEC

SEQ ID NO: 149 - protein, 17 aa, synthetic construct
AIYPDNGDTSYNQRFKV

SEQ ID NO: 150 - protein, 11 aa, synthetic construct
RASENIYGALN

SEQ ID NO: 151 - protein, 30 aa, synthetic construct
QVQLVQSGAEVKKPGASVKVSCKASGYTFT

SEQ ID NO: 152 - protein, 30 aa, synthetic construct
QVQLVQSGAEVKKPGASVKVSCKASGYIFT

SEQ ID NO: 153 - protein, 30 aa, synthetic construct
QVQLVQSGAEVKKPGASVKVSCKASGYIFR

SEQ ID NO: 154 - protein, 14 aa, synthetic construct
WVRQAPGQGLEWMG

SEQ ID NO: 155 - protein, 14 aa, synthetic construct
WVKQAPGQGLEWMG

SEQ ID NO: 156 - protein, 32 aa, synthetic construct
RATLTADTSTSTVYMELSSLRSEDTAVYYCAR

SEQ ID NO: 157 - protein, 11 aa, synthetic construct
WGQGTTVTVSS

SEQ ID NO: 158 - protein, 23 aa, synthetic construct
DIQMTQSPSSLSASVGDRVTITC

SEQ ID NO: 159 - protein, 15 aa, synthetic construct
WYQQKPGKAPKLLIY

SEQ ID NO: 160 - protein, 15 aa, synthetic construct
WYQRKPGKAPKLLIY

SEQ ID NO: 161 - protein, 15 aa, synthetic construct
WYQRKPGKSPKLLIY

SEQ ID NO: 162 - protein, 32 aa, synthetic construct
GVPSRFSGSGSGTDFTLTISSLQPEDFATYYC

SEQ ID NO: 163 - protein, 32 aa, synthetic construct
GVPSRFSGSGSGTDYTLTISSLQPEDVATYYC

SEQ ID NO: 164 - protein, 32 aa, synthetic construct
GVPSRFSGSGSGTDYTLTISSLQPEDFATYYC

SEQ ID NO: 165 - protein, 10 aa, synthetic construct
FGGGTKVEIK

SEQ ID NO: 166 - protein, 10 aa, synthetic construct
FGGGTKLEIK

SEQ ID NO: 167 - protein, 113 aa, synthetic construct
QVQLVQSGAEVKKPGASVKVSCKASGYTFTNYYIHWVRQAPGQGLEWMGAIYPDNGDTSYNQRFKVRATLTADTSTSTVYMELSSLRSEDTAVYYCARAFTYWGQGTTVTVSS

SEQ ID NO: 168 - protein, 113 aa, synthetic construct
QVQLVQSGAEVKKPGASVKVSCKASGYIFTNYYIHWVRQAPGQGLEWMGAIYPDNGDTSYNQRFKVRATLTADTSTSTVYMELSSLRSEDTAVYYCARAFTYWGQGTTVTVSS

SEQ ID NO: 169 - protein, 113 aa, synthetic construct
QVQLVQSGAEVKKPGASVKVSCKASGYIFRNYYIHWVRQAPGQGLEWMGAIYPDNGDTSYNQRFKVRATLTADTSTSTVYMELSSLRSEDTAVYYCARAFTYWGQGTTVTVSS

SEQ ID NO: 170 - protein, 113 aa, synthetic construct
QVQLVQSGAEVKKPGASVKVSCKASGYIFRNYYIHWVKQAPGQGLEWMGAIYPDNGDTSYNQRFKVRATLTADTSTSTVYMELSSLRSEDTAVYYCARAFTYWGQGTTVTVSS

SEQ ID NO: 171 - protein, 107 aa, synthetic construct
DIQMTQSPSSLSASVGDRVTITCRASENIYGALNWYQQKPGKAPKLLIYGATNLADGVPSRFSGSGSGTDFTLTISSLQPEDFATYYCQNVLSTPYTFGGGTKVEIK

SEQ ID NO: 172 - protein, 107 aa, synthetic construct
DIQMTQSPSSLSASVGDRVTITCGASENIYGALNWYQQKPGKAPKLLIYGATNLADGVPSRFSGSGSGTDYTLTISSLQPEDVATYYCQNVLSTPYTFGGGTKVEIK

SEQ ID NO: 173 - protein, 107 aa, synthetic construct
DIQMTQSPSSLSASVGDRVTITCGASENIYGALNWYQRKPGKAPKLLIYGATNLADGVPSRFSGSGSGTDYTLTISSLQPEDFATYYCQNVLSTPYTFGGGTKLEIK

SEQ ID NO: 174 - protein, 107 aa, synthetic construct
DIQMTQSPSSLSASVGDRVTITCGASENIYGALNWYQRKPGKSPKLLIYGATNLADGVPSRFSGSGSGTDYTLTISSLQPEDVATYYCQNVLSTPYTFGGGTKLEIK

SEQ ID NO: 175 - protein, 30 aa, synthetic construct; identical to SEQ ID NO: 151

SEQ ID NO: 176 - protein, 30 aa, synthetic construct
QVQLVQSGAEVKKPGASVKVSCKASGYTFS

SEQ ID NO: 177 - protein, 14 aa, synthetic construct
WVRQAPGQGLEWMG

SEQ ID NO: 178 - protein, 14 aa, synthetic construct
WVRQAPGQGLEWIG

SEQ ID NO: 179 - protein, 14 aa, synthetic construct
WVKQAPGQGLEWIG

SEQ ID NO: 180 - protein, 32 aa, synthetic construct; identical to SEQ ID NO: 156

SEQ ID NO: 181 - protein, 11 aa, synthetic construct
WGQGTTVTVSS

SEQ ID NO: 182 - protein, 23 aa, synthetic construct
DIQMTQSPSSLSASVGDRVTITC

SEQ ID NO: 183 - protein, 15 aa, synthetic construct
WYQQKPGKAPKLLIY

SEQ ID NO: 184 - protein, 15 aa, synthetic construct
WYQQKPGKSPKLLIY

SEQ ID NO: 185 - protein, 15 aa, synthetic construct
WYQQKPGKSPKLLVY

SEQ ID NO: 186 - protein, 32 aa, synthetic construct; identical to SEQ ID NO: 162

SEQ ID NO: 187 - protein, 32 aa, synthetic construct; identical to SEQ ID NO: 164

SEQ ID NO: 188 - protein, 10 aa, synthetic construct
FGGGTKVEIK

SEQ ID NO: 189 - protein, 10 aa, synthetic construct
FGGGTKLEIK

SEQ ID NO: 190 - protein, 114 aa, synthetic construct
QVQLVQSGAEVKKPGASVKVSCKASGYTFTFYNMHWVRQAPGQGLEWMGLIYPDNGDTSYNQKFKGRATLTADTSTSTVYMELSSLRSEDTAVYYCARGGLDYWGQGTTVTVSS

SEQ ID NO: 191 - protein, 114 aa, synthetic construct
QVQLVQSGAEVKKPGASVKVSCKASGYTFTFYNMHWVRQAPGQGLEWIGLIYPDNGDTSYNQKFKGRATLTADTSTSTVYMELSSLRSEDTAVYYCARGGLDYWGQGTTVTVSS

SEQ ID NO: 192 - protein, 114 aa, synthetic construct
QVQLVQSGAEVKKPGASVKVSCKASGYTFSFYNMHWVRQAPGQGLEWIGLIYPDNGDTSYNQKFKGRATLTADTSTSTVYMELSSLRSEDTAVYYCARGGLDYWGQGTTVTVSS

SEQ ID NO: 193 - protein, 114 aa, synthetic construct
QVQLVQSGAEVKKPGASVKVSCKASGYTFSFYNMHWVKQAPGQGLEWIGLIYPDNGDTSYNQKFKGRATLTADTSTSTVYMELSSLRSEDTAVYYCARGGLDYWGQGTTVTVSS

SEQ ID NO: 194 - protein, 107 aa, synthetic construct
DIQMTQSPSSLSASVGDRVTITCRASENIYSNLAWYQQKPGKAPKLLIYAATNLADGVPSRFSGSGSGTDFTLTISSLQPEDFATYYCQHFWGTPYTFGGGTKVEIK

SEQ ID NO: 195 - protein, 107 aa, synthetic construct
DIQMTQSPSSLSASVGDRVTITCRASENIYSNLAWYQQKPGKSPKLLIYAATNLADGVPSRFSGSGSGTDYTLTISSLQPEDFATYYCQHFWGTPYTFGGGTKVEIK

SEQ ID NO: 196 - protein, 107 aa, synthetic construct
DIQMTQSPSSLSASVGDRVTITCRASENIYSNLAWYQQKPGKSPKLLVYAATNLADGVPSRFSGSGSGTDYTLTISSLQPEDFATYYCQHFWGTPYTFGGGTKVEIK

SEQ ID NO: 197 - protein, 107 aa, synthetic construct
DIQMTQSPSSLSASVGDRVTITCRASENIYSNLAWYQQKPGKSPKLLVYAATNLADGVPSRFSGSGSGTDYTLTISSLQPEDFATYYCQHFWGTPYTFGGGTKLEIK

SEQ ID NO: 198 - protein, 443 aa, synthetic construct
EIQLQQSGAELVKPGASVKMSCKASGYIFRNYYIHWVKRTPGQGLEWIGAIYPDNGDTSYNQRFKVKATLTADTSSSTAYMQLSSLTSEDSAVYYCARAFTYWGQGTTLTVSSASTKGPSVFPLAPSSKSTSGGTAALGCLVKDYFPEPVTVSWNSGALTSGVHTFPAVLQSSGLYSLSSVVTVPSSSLGTQTYICNVNHKPSNTKVDKKVEPKSCDKTHTCPPCPAPELLGGPSVFLFPPKPKDTLMISRTPEVTCVVVDVSHEDPEVKFNWYVDGVEVHNAKTKPREEQYNSTYRVVSVLTVLHQDWLNGKEYKCKVSNKALPAPIEKTISKAKGQPREPQVYTLPPSREEMTKNQVSLTCLVKGFYPSDIAVEWESNGQPENNYKTTPPVLDSDGSFFLYSKLTVDKSRWQQGNVFSCSVMHEALHNHYTQKSLSLSPGK